European Patent Application EP 4 474 476 A1, published December 11, 2024. Title: Ｔ細胞の製造方法. Applicant: 国立大学法人京都大学. The sequence listing filed with the application follows.

SEQUENCE LISTING (10 sequences)

SEQ ID NO: 1 - DNA, 1191 bp, Homo sapiens
  source 1..1191: mol_type = other DNA
atgcccaaccccaggcctggcaagccctcggccccttccttggcccttggcccatccccaggagcctcgcccagctggagggctgcacccaaagcctcagacctgctgggggcccggggcccagggggaaccttccagggccgagatcttcgaggcggggcccatgcctcctcttcttccttgaaccccatgccaccatcgcagctgcagctctcaacggtggatgcccacgcccggacccctgtgctgcaggtgcaccccctggagagcccagccatgatcagcctcacaccacccaccaccgccactggggtcttctccctcaaggcccggcctggcctcccacctgggatcaacgtggccagcctggaatgggtgtccagggagccggcactgctctgcaccttcccaaatcccagtgcacccaggaaggacagcaccctttcggctgtgccccagagctcctacccactgctggcaaatggtgtctgcaagtggcccggatgtgagaaggtcttcgaagagccagaggacttcctcaagcactgccaggcggaccatcttctggatgagaagggcagggcacaatgtctcctccagagagagatggtacagtctctggagcagcagctggtgctggagaaggagaagctgagtgccatgcaggcccacctggctgggaaaatggcactgaccaaggcttcatctgtggcatcatccgacaagggctcctgctgcatcgtagctgctggcagccaaggccctgtcgtcccagcctggtctggcccccgggaggcccctgacagcctgtttgctgtccggaggcacctgtggggtagccatggaaacagcacattcccagagttcctccacaacatggactacttcaagttccacaacatgcgaccccctttcacctacgccacgctcatccgctgggccatcctggaggctccagagaagcagcggacactcaatgagatctaccactggttcacacgcatgtttgccttcttcagaaaccatcctgccacctggaagaacgccatccgccacaacctgagtctgcacaagtgctttgtgcgggtggagagcgagaagggggctgtgtggaccgtggatgagctggagttccgcaagaaacggagccagaggcccagcaggtgttccaaccctacacctggcccctga

SEQ ID NO: 2 - DNA, 1296 bp, Homo sapiens
  source 1..1296: mol_type = other DNA
atgcccaaccccaggcctggcaagccctcggccccttccttggcccttggcccatccccaggagcctcgcccagctggagggctgcacccaaagcctcagacctgctgggggcccggggcccagggggaaccttccagggccgagatcttcgaggcggggcccatgcctcctcttcttccttgaaccccatgccaccatcgcagctgcagctgcccacactgcccctagtcatggtggcaccctccggggcacggctgggccccttgccccacttacaggcactcctccaggacaggccacatttcatgcaccagctctcaacggtggatgcccacgcccggacccctgtgctgcaggtgcaccccctggagagcccagccatgatcagcctcacaccacccaccaccgccactggggtcttctccctcaaggcccggcctggcctcccacctgggatcaacgtggccagcctggaatgggtgtccagggagccggcactgctctgcaccttcccaaatcccagtgcacccaggaaggacagcaccctttcggctgtgccccagagctcctacccactgctggcaaatggtgtctgcaagtggcccggatgtgagaaggtcttcgaagagccagaggacttcctcaagcactgccaggcggaccatcttctggatgagaagggcagggcacaatgtctcctccagagagagatggtacagtctctggagcagcagctggtgctggagaaggagaagctgagtgccatgcaggcccacctggctgggaaaatggcactgaccaaggcttcatctgtggcatcatccgacaagggctcctgctgcatcgtagctgctggcagccaaggccctgtcgtcccagcctggtctggcccccgggaggcccctgacagcctgtttgctgtccggaggcacctgtggggtagccatggaaacagcacattcccagagttcctccacaacatggactacttcaagttccacaacatgcgaccccctttcacctacgccacgctcatccgctgggccatcctggaggctccagagaagcagcggacactcaatgagatctaccactggttcacacgcatgtttgccttcttcagaaaccatcctgccacctggaagaacgccatccgccacaacctgagtctgcacaagtgctttgtgcgggtggagagcgagaagggggctgtgtggaccgtggatgagctggagttccgcaagaaacggagccagaggcccagcaggtgttccaaccctacacctggcccctga

SEQ ID NO: 3 - protein, 396 aa, Homo sapiens
MPNPRPGKPSAPSLALGPSPGASPSWRAAPKASDLLGARGPGGTFQGRDLRGGAHASSSSLNPMPPSQLQLSTVDAHARTPVLQVHPLESPAMISLTPPTTATGVFSLKARPGLPPGINVASLEWVSREPALLCTFPNPSAPRKDSTLSAVPQSSYPLLANGVCKWPGCEKVFEEPEDFLKHCQADHLLDEKGRAQCLLQREMVQSLEQQLVLEKEKLSAMQAHLAGKMALTKASSVASSDKGSCCIVAAGSQGPVVPAWSGPREAPDSLFAVRRHLWGSHGNSTFPEFLHNMDYFKFHNMRPPFTYATLIRWAILEAPEKQRTLNEIYHWFTRMFAFFRNHPATWKNAIRHNLSLHKCFVRVESEKGAVWTVDELEFRKKRSQRPSRCSNPTPGP

SEQ ID NO: 4 - protein, 431 aa, Homo sapiens
MPNPRPGKPSAPSLALGPSPGASPSWRAAPKASDLLGARGPGGTFQGRDLRGGAHASSSSLNPMPPSQLQLPTLPLVMVAPSGARLGPLPHLQALLQDRPHFMHQLSTVDAHARTPVLQVHPLESPAMISLTPPTTATGVFSLKARPGLPPGINVASLEWVSREPALLCTFPNPSAPRKDSTLSAVPQSSYPLLANGVCKWPGCEKVFEEPEDFLKHCQADHLLDEKGRAQCLLQREMVQSLEQQLVLEKEKLSAMQAHLAGKMALTKASSVASSDKGSCCIVAAGSQGPVVPAWSGPREAPDSLFAVRRHLWGSHGNSTFPEFLHNMDYFKFHNMRPPFTYATLIRWAILEAPEKQRTLNEIYHWFTRMFAFFRNHPATWKNAIRHNLSLHKCFVRVESEKGAVWTVDELEFRKKRSQRPSRCSNPTPGP

SEQ ID NO: 5 - DNA, 238 bp, Homo sapiens
  source 1..238: mol_type = other DNA
taggttagtctttttttctgtggcttctgtctctggttttgtgcttagaaagtcctttcctacttgaaaatgagataaatgttcacctatgttggcttctagtctcttttatggcttcattttttccatttactatagaggttaagagtgtgggtactggagccagactgtctgggacaaacccagcgtcaccccaagccctatgtgtgatttttagccaggcacttaacctctccat

SEQ ID NO: 6 - DNA, 360 bp, Homo sapiens
  source 1..360: mol_type = other DNA
ccaagaagggccaggtcttcagagctaggggcttgtcatagtggccagatggacatcacctaccacatccaccagcacccatgtcaccccacctgggccaagcctgctgcaggacagggcagccagttctcggaacgaaacctgtggggtggggtatctgccctcttctcttcctccgtggtgtcgatgaagcccggcgcatccggccgccatgacgtcaatggcggaaaaatctgggcaagtcgggggctgtgacaacagggcccagatgcagaccccgatatgaaaacataatctgtgtcccagaaacatcccccattcagcttctgagaaacccagtcagaaagggacgtcccaaca

SEQ ID NO: 7 - DNA, 218 bp, Homo sapiens
  source 1..218: mol_type = other DNA
gaggccctgggcccaggatggggcaggcagggtggggtacctggacctacaggtgccgacctttactgtggcactgggcgggaggggggctggctggggcacaggaagtggtttctgggtcccaggcaagtctgtgacttatgcagatgttgcagggccaagaaaatccccacctgccaggcctcagagattggaggctctccccgacctcccaatcc

SEQ ID NO: 8 - DNA, 383 bp, Homo sapiens
  source 1..383: mol_type = other DNA
tcccatccacacatagagcttcagattctctttctttccccagagaccctcaaatatcctctcactcacagaatggtgtctctgcctgcctcgggttggccctgtgatttattttagttcttttcccttgttttttttttttcaaactctatacacttttgttttaaaaactgtggtttctcatgagccctattatctcattgatacctctcacctctgtggtgaggggaagaaatcatattttcagatgactcgtaaagggcaaagaaaaaaacccaaaatttcaaaatttccgtttaagtctcataatcaagaaaaggagaaacacagagagagagaaaaaaaaaactatgagaacccctccccaccccgtgattatcagc

SEQ ID NO: 9 - protein, 965 aa, synthetic construct
MDWTWRILFLVAAATGAHSDIQMTQTTSSLSASLGDRVTISCRASQDISKYLNWYQQKPDGTVKLLIYHTSRLHSGVPSRFSGSGSGTDYSLTISNLEQEDIATYFCQQGNTLPYTFGGGTKLEITGGGGSGGGGSGGGGSEVKLQESGPGLVAPSQSLSVTCTVSGVSLPDYGVSWIRQPPRKGLEWLGVIWGSETTYYNSALKSRLTIIKDNSKSQVFLKMNSLQTDDTAIYYCAKHYYYGGSYAMDYWGQGTSVTVSSFVPVFLPAKPTTTPAPRPPTPAPTIASQPLSLRPEACRPAAGGAVHTRGLDFACDIYIWAPLAGTCGVLLLSLVITLYCNHRNRSKRSRLLHSDYMNMTPRRPGPTRKHYQPYAPPRDFAAYRSHTNNKIEKIYIMKADTVIVGTVKAELPEGRGLAGPAEPELEEELEADHTPHYPEQETEPPLGSCSDVMLSVEEEGKEDPLPTAASGKRVKFSRSADAPAYQQGQNQLYNELNLGRREEYDVLDKRRGRDPEMGGKPRRKNPQEGLYNELQKDKMAEAYSEIGMKGERRRGKGHDGLYQGLSTATKDTYDALHMQALPPRLEGGGEGRGSLLTCGDVEENPGPRMLLLVTSLLLCELPHPAFLLIPRKVCNGIGIGEFKDSLSINATNIKHFKNCTSISGDLHILPVAFRGDSFTHTPPLDPQELDILKTVKEITGFLLIQAWPENRTDLHAFENLEIIRGRTKQHGQFSLAVVSLNITSLGLRSLKEISDGDVIISGNKNLCYANTINWKKLFGTSGQKTKIISNRGENSCKATGQVCHALCSPEGCWGPEPRDCVSCRNVSRGRECVDKCNLLEGEPREFVENSECIQCHPECLPQAMNITCTGRGPDNCIQCAHYIDGPHCVKTCPAGVMGENNTLVWKYADAGHVCHLCHPNCTYGCTGPGLEGCPTNGPKIPSIATGMVGALLLLLVVALGIGLFM

SEQ ID NO: 10 - protein, 400 aa, Homo sapiens
MYRMQLLSCIALSLALVTNSATSNWVNVISDLKKIEDLIQSMHIDATLYTESDVHPSCKVTAMKCFLLELQVISLESGDASIHDTVENLIILANNSLSSNGNVTESGCKECEELEEKNIKEFLQSFVHIVQMFINTSSGGGSGGGGSGGGGSGGGGSGGGSLQITCPPPMSVEHADIWVKSYSLYSRERYICNSGFKRKAGTSSLTECVLNKATNVAHWTTPSLKCIRDPALVHQRPAPPSTVTTAGVTPQPESLSPSGKEPAASSPSSNNTAATTAAIVPGSQLMPSKSPSTGTTEISSHESSHGTPSQTTAKNWELTASASHQPPGVYPQGHSDTTVAISTSTVLLCGLSAVSLLACYLKSRQTPPLASVEMEAMEALPVTWGTSSRDEDLENCSHHL